European Patent Specification EP 3 980 777 B1, published February 25, 2026. Title: METHODS FOR MANUFACTURING T CELLS BY DIRECT SORTING AND COMPOSITIONS THEREOF. Applicant: Immatics US, Inc. The sequence listing filed with the application follows.

SEQUENCE LISTING (161 sequences)

SEQ ID NO: 1 - protein, 10 aa, Homo sapiens
YLYDSETKNA

SEQ ID NO: 2 - protein, 9 aa, Homo sapiens
HLMDQPLSV

SEQ ID NO: 3 - protein, 9 aa, Homo sapiens
GLLKKINSV

SEQ ID NO: 4 - protein, 9 aa, Homo sapiens
FLVDGSSAL

SEQ ID NO: 5 - protein, 10 aa, Homo sapiens
FLFDGSANLV

SEQ ID NO: 6 - protein, 9 aa, Homo sapiens
FLYKIIDEL

SEQ ID NO: 7 - protein, 11 aa, Homo sapiens
FILDSAETTTL

SEQ ID NO: 8 - protein, 9 aa, Homo sapiens
SVDVSPPKV

SEQ ID NO: 9 - protein, 8 aa, Homo sapiens
VADKIHSV

SEQ ID NO: 10 - protein, 9 aa, Homo sapiens
IVDDLTINL

SEQ ID NO: 11 - protein, 9 aa, Homo sapiens
GLLEELVTV

SEQ ID NO: 12 - protein, 10 aa, Homo sapiens
TLDGAAVNQV

SEQ ID NO: 13 - protein, 10 aa, Homo sapiens
SVLEKEIYSI

SEQ ID NO: 14 - protein, 9 aa, Homo sapiens
LLDPKTIFL

SEQ ID NO: 15 - protein, 9 aa, Homo sapiens
YTFSGDVQL

SEQ ID NO: 16 - protein, 9 aa, Homo sapiens
YLMDDFSSL

SEQ ID NO: 17 - protein, 9 aa, Homo sapiens
KVWSDVTPL

SEQ ID NO: 18 - protein, 11 aa, Homo sapiens
LLWGHPRVALA

SEQ ID NO: 19 - protein, 11 aa, Homo sapiens
KIWEELSVLEV

SEQ ID NO: 20 - protein, 9 aa, Homo sapiens
LLIPFTIFM

SEQ ID NO: 21 - protein, 9 aa, Homo sapiens
FLIENLLAA

SEQ ID NO: 22 - protein, 11 aa, Homo sapiens
LLWGHPRVALA

SEQ ID NO: 23 - protein, 9 aa, Homo sapiens
FLLEREQLL

SEQ ID NO: 24 - protein, 9 aa, Homo sapiens
SLAETIFIV

SEQ ID NO: 25 - protein, 9 aa, Homo sapiens
TLLEGISRA

SEQ ID NO: 26 - protein, 9 aa, Homo sapiens
ILQDGQFLV

SEQ ID NO: 27 - protein, 10 aa, Homo sapiens
VIFEGEPMYL

SEQ ID NO: 28 - protein, 9 aa, Homo sapiens
SLFESLEYL

SEQ ID NO: 29 - protein, 9 aa, Homo sapiens
SLLNQPKAV

SEQ ID NO: 30 - protein, 9 aa, Homo sapiens
GLAEFQENV

SEQ ID NO: 31 - protein, 9 aa, Homo sapiens
KLLAVIHEL

SEQ ID NO: 32 - protein, 9 aa, Homo sapiens
TLHDQVHLL

SEQ ID NO: 33 - protein, 11 aa, Homo sapiens
TLYNPERTITV

SEQ ID NO: 34 - protein, 9 aa, Homo sapiens
KLQEKIQEL

SEQ ID NO: 35 - protein, 10 aa, Homo sapiens
SVLEKEIYSI

SEQ ID NO: 36 - protein, 11 aa, Homo sapiens
RVIDDSLVVGV

SEQ ID NO: 37 - protein, 9 aa, Homo sapiens
VLFGELPAL

SEQ ID NO: 38 - protein, 9 aa, Homo sapiens
GLVDIMVHL

SEQ ID NO: 39 - protein, 9 aa, Homo sapiens
FLNAIETAL

SEQ ID NO: 40 - protein, 9 aa, Homo sapiens
ALLQALMEL

SEQ ID NO: 41 - protein, 9 aa, Homo sapiens
ALSSSQAEV

SEQ ID NO: 42 - protein, 11 aa, Homo sapiens
SLITGQDLLSV

SEQ ID NO: 43 - protein, 9 aa, Homo sapiens
QLIEKNWLL

SEQ ID NO: 44 - protein, 9 aa, Homo sapiens
LLDPKTIFL

SEQ ID NO: 45 - protein, 9 aa, Homo sapiens
RLHDENILL

SEQ ID NO: 46 - protein, 9 aa, Homo sapiens
YTFSGDVQL

SEQ ID NO: 47 - protein, 9 aa, Homo sapiens
GLPSATTTV

SEQ ID NO: 48 - protein, 11 aa, Homo sapiens
GLLPSAESIKL

SEQ ID NO: 49 - protein, 9 aa, Homo sapiens
KTASINQNV

SEQ ID NO: 50 - protein, 9 aa, Homo sapiens
SLLQHLIGL

SEQ ID NO: 51 - protein, 9 aa, Homo sapiens
YLMDDFSSL

SEQ ID NO: 52 - protein, 9 aa, Homo sapiens
LMYPYIYHV

SEQ ID NO: 53 - protein, 9 aa, Homo sapiens
KVWSDVTPL

SEQ ID NO: 54 - protein, 11 aa, Homo sapiens
LLWGHPRVALA

SEQ ID NO: 55 - protein, 9 aa, Homo sapiens
VLDGKVAVV

SEQ ID NO: 56 - protein, 9 aa, Homo sapiens
GLLGKVTSV

SEQ ID NO: 57 - protein, 9 aa, Homo sapiens
KMISAIPTL

SEQ ID NO: 58 - protein, 11 aa, Homo sapiens
GLLETTGLLAT

SEQ ID NO: 59 - protein, 9 aa, Homo sapiens
TLNTLDINL

SEQ ID NO: 60 - protein, 9 aa, Homo sapiens
VIIKGLEEI

SEQ ID NO: 61 - protein, 9 aa, Homo sapiens
YLEDGFAYV

SEQ ID NO: 62 - protein, 11 aa, Homo sapiens
KIWEELSVLEV

SEQ ID NO: 63 - protein, 9 aa, Homo sapiens
LLIPFTIFM

SEQ ID NO: 64 - protein, 10 aa, Homo sapiens
ISLDEVAVSL

SEQ ID NO: 65 - protein, 10 aa, Homo sapiens
KISDFGLATV

SEQ ID NO: 66 - protein, 11 aa, Homo sapiens
KLIGNIHGNEV

SEQ ID NO: 67 - protein, 9 aa, Homo sapiens
ILLSVLHQL

SEQ ID NO: 68 - protein, 9 aa, Homo sapiens
LDSEALLTL

SEQ ID NO: 69 - protein, 13 aa, Homo sapiens
VLQENSSDYQSNL

SEQ ID NO: 70 - protein, 11 aa, Homo sapiens
HLLGEGAFAQV

SEQ ID NO: 71 - protein, 9 aa, Homo sapiens
SLVENIHVL

SEQ ID NO: 72 - protein, 9 aa, Homo sapiens
YTFSGDVQL

SEQ ID NO: 73 - protein, 9 aa, Homo sapiens
SLSEKSPEV

SEQ ID NO: 74 - protein, 10 aa, Homo sapiens
AMFPDTIPRV

SEQ ID NO: 75 - protein, 9 aa, Homo sapiens
FLIENLLAA

SEQ ID NO: 76 - protein, 9 aa, Homo sapiens
FTAEFLEKV

SEQ ID NO: 77 - protein, 9 aa, Homo sapiens
ALYGNVQQV

SEQ ID NO: 78 - protein, 9 aa, Homo sapiens
LFQSRIAGV

SEQ ID NO: 79 - protein, 11 aa, Homo sapiens
ILAEEPIYIRV

SEQ ID NO: 80 - protein, 9 aa, Homo sapiens
FLLEREQLL

SEQ ID NO: 81 - protein, 10 aa, Homo sapiens
LLLPLELSLA

SEQ ID NO: 82 - protein, 9 aa, Homo sapiens
SLAETIFIV

SEQ ID NO: 83 - protein, 11 aa, Homo sapiens
AILNVDEKNQV

SEQ ID NO: 84 - protein, 9 aa, Homo sapiens
RLFEEVLGV

SEQ ID NO: 85 - protein, 9 aa, Homo sapiens
YLDEVAFML

SEQ ID NO: 86 - protein, 11 aa, Homo sapiens
KLIDEDEPLFL

SEQ ID NO: 87 - protein, 9 aa, Homo sapiens
KLFEKSTGL

SEQ ID NO: 88 - protein, 11 aa, Homo sapiens
SLLEVNEASSV

SEQ ID NO: 89 - protein, 10 aa, Homo sapiens
GVYDGREHTV

SEQ ID NO: 90 - protein, 10 aa, Homo sapiens
GLYPVTLVGV

SEQ ID NO: 91 - protein, 9 aa, Homo sapiens
ALLSSVAEA

SEQ ID NO: 92 - protein, 9 aa, Homo sapiens
TLLEGISRA

SEQ ID NO: 93 - protein, 9 aa, Homo sapiens
SLIEESEEL

SEQ ID NO: 94 - protein, 9 aa, Homo sapiens
ALYVQAPTV

SEQ ID NO: 95 - protein, 10 aa, Homo sapiens
KLIYKDLVSV

SEQ ID NO: 96 - protein, 9 aa, Homo sapiens
ILQDGQFLV

SEQ ID NO: 97 - protein, 9 aa, Homo sapiens
SLLDYEVSI

SEQ ID NO: 98 - protein, 9 aa, Homo sapiens
LLGDSSFFL

SEQ ID NO: 99 - protein, 10 aa, Homo sapiens
VIFEGEPMYL

SEQ ID NO: 100 - protein, 9 aa, Homo sapiens
ALSYILPYL

SEQ ID NO: 101 - protein, 9 aa, Homo sapiens
FLFVDPELV

SEQ ID NO: 102 - protein, 11 aa, Homo sapiens
SEWGSPHAAVP

SEQ ID NO: 103 - protein, 9 aa, Homo sapiens
ALSELERVL

SEQ ID NO: 104 - protein, 9 aa, Homo sapiens
SLFESLEYL

SEQ ID NO: 105 - protein, 9 aa, Homo sapiens
KVLEYVIKV

SEQ ID NO: 106 - protein, 10 aa, Homo sapiens
VLLNEILEQV

SEQ ID NO: 107 - protein, 9 aa, Homo sapiens
SLLNQPKAV

SEQ ID NO: 108 - protein, 9 aa, Homo sapiens
KMSELQTYV

SEQ ID NO: 109 - protein, 11 aa, Homo sapiens
ALLEQTGDMSL

SEQ ID NO: 110 - protein, 11 aa, Homo sapiens
VIIKGLEEITV

SEQ ID NO: 111 - protein, 9 aa, Homo sapiens
KQFEGTVEI

SEQ ID NO: 112 - protein, 9 aa, Homo sapiens
KLQEEIPVL

SEQ ID NO: 113 - protein, 9 aa, Homo sapiens
GLAEFQENV

SEQ ID NO: 114 - protein, 9 aa, Homo sapiens
NVAEIVIHI

SEQ ID NO: 115 - protein, 9 aa, Homo sapiens
ALAGIVTNV

SEQ ID NO: 116 - protein, 12 aa, Homo sapiens
NLLIDDKGTIKL

SEQ ID NO: 117 - protein, 10 aa, Homo sapiens
VLMQDSRLYL

SEQ ID NO: 118 - protein, 9 aa, Homo sapiens
KVLEHVVRV

SEQ ID NO: 119 - protein, 9 aa, Homo sapiens
LLWGNLPEI

SEQ ID NO: 120 - protein, 9 aa, Homo sapiens
SLMEKNQSL

SEQ ID NO: 121 - protein, 9 aa, Homo sapiens
KLLAVIHEL

SEQ ID NO: 122 - protein, 10 aa, Homo sapiens
ALGDKFLLRV

SEQ ID NO: 123 - protein, 11 aa, Homo sapiens
FLMKNSDLYGA

SEQ ID NO: 124 - protein, 10 aa, Homo sapiens
KLIDHQGLYL

SEQ ID NO: 125 - protein, 12 aa, Homo sapiens
GPGIFPPPPPQP

SEQ ID NO: 126 - protein, 9 aa, Homo sapiens
ALNESLVEC

SEQ ID NO: 127 - protein, 9 aa, Homo sapiens
GLAALAVHL

SEQ ID NO: 128 - protein, 9 aa, Homo sapiens
LLLEAVWHL

SEQ ID NO: 129 - protein, 9 aa, Homo sapiens
SIIEYLPTL

SEQ ID NO: 130 - protein, 9 aa, Homo sapiens
TLHDQVHLL

SEQ ID NO: 131 - protein, 9 aa, Homo sapiens
SLLMWITQC

SEQ ID NO: 132 - protein, 11 aa, Homo sapiens
FLLDKPQDLSI

SEQ ID NO: 133 - protein, 10 aa, Homo sapiens
YLLDMPLWYL

SEQ ID NO: 134 - protein, 9 aa, Homo sapiens
GLLDCPIFL

SEQ ID NO: 135 - protein, 9 aa, Homo sapiens
VLIEYNFSI

SEQ ID NO: 136 - protein, 11 aa, Homo sapiens
TLYNPERTITV

SEQ ID NO: 137 - protein, 9 aa, Homo sapiens
AVPPPPSSV

SEQ ID NO: 138 - protein, 9 aa, Homo sapiens
KLQEELNKV

SEQ ID NO: 139 - protein, 11 aa, Homo sapiens
KLMDPGSLPPL

SEQ ID NO: 140 - protein, 9 aa, Homo sapiens
ALIVSLPYL

SEQ ID NO: 141 - protein, 9 aa, Homo sapiens
FLLDGSANV

SEQ ID NO: 142 - protein, 10 aa, Homo sapiens
ALDPSGNQLI

SEQ ID NO: 143 - protein, 9 aa, Homo sapiens
ILIKHLVKV

SEQ ID NO: 144 - protein, 9 aa, Homo sapiens
VLLDTILQL

SEQ ID NO: 145 - protein, 9 aa, Homo sapiens
HLIAEIHTA

SEQ ID NO: 146 - protein, 9 aa, Homo sapiens
SMNGGVFAV

SEQ ID NO: 147 - protein, 9 aa, Homo sapiens
MLAEKLLQA

SEQ ID NO: 148 - protein, 9 aa, Homo sapiens
YMLDIFHEV

SEQ ID NO: 149 - protein, 11 aa, Homo sapiens
ALWLPTDSATV

SEQ ID NO: 150 - protein, 9 aa, Homo sapiens
GLASRILDA

SEQ ID NO: 151 - protein, 9 aa, Homo sapiens
ALSVLRLAL

SEQ ID NO: 152 - protein, 9 aa, Homo sapiens
SYVKVLHHL

SEQ ID NO: 153 - protein, 9 aa, Homo sapiens
VYLPKIPSW

SEQ ID NO: 154 - protein, 9 aa, Homo sapiens
NYEDHFPLL

SEQ ID NO: 155 - protein, 9 aa, Homo sapiens
VYIAELEKI

SEQ ID NO: 156 - protein, 12 aa, Homo sapiens
VHFEDTGKTLLF

SEQ ID NO: 157 - protein, 9 aa, Homo sapiens
VLSPFILTL

SEQ ID NO: 158 - protein, 9 aa, Homo sapiens
HLLEGSVGV

SEQ ID NO: 159 - protein, 9 aa, Homo sapiens
ALREEEEGV

SEQ ID NO: 160 - protein, 10 aa, Homo sapiens
KEADPTGHSY

SEQ ID NO: 161 - protein, 9 aa, Homo sapiens
TLDEKVAEL